European Patent Specification EP 3 221 330 B1, published April 22, 2026. Title: PHOSPHORAMIDITE SYNTHONES FOR THE SYNTHESIS OF SELF-NEUTRALIZING OLIGONUCLEOTIDE COMPOUNDS. Applicant: Tabatadze, David Yanachkov, Ivan. The sequence listing filed with the application follows.

SEQUENCE LISTING (31 sequences)

SEQ ID NO: 1 - DNA, 19 bp, Artificial Sequence
  Synthetic
atagtagtagtcctagtct

SEQ ID NO: 2 - DNA, 19 bp, Artificial Sequence
  Synthetic
atagtagtagtcctagtct

SEQ ID NO: 3 - DNA, 19 bp, Artificial Sequence
  Synthetic
atagtagtagtcctagtct

SEQ ID NO: 4 - RNA, 19 nt, Artificial Sequence
  Synthetic
uucguaguugucuuagucc

SEQ ID NO: 5 - RNA, 19 nt, Artificial Sequence
  Synthetic
uucguaguugucuuagucc

SEQ ID NO: 6 - RNA, 19 nt, Artificial Sequence
  Synthetic
uucguaguugucuuagucc

SEQ ID NO: 7 - RNA, 19 nt, Artificial Sequence
  Synthetic
uucguaguugucuuagucc

SEQ ID NO: 8 - RNA, 19 nt, Artificial Sequence
  Synthetic
uucguaguugucuuagucc

SEQ ID NO: 9 - RNA, 19 nt, Artificial Sequence
  Synthetic
uucguaguugucuuagucc

SEQ ID NO: 10 - RNA, 19 nt, Artificial Sequence
  Synthetic
uucguaguugucuuagucc

SEQ ID NO: 11 - RNA, 21 nt, Artificial Sequence
  Synthetic
ucguacuuaucuuaauccuac

SEQ ID NO: 12 - RNA, 21 nt, Artificial Sequence
  Synthetic
ucguacuuaucuuaauccuac

SEQ ID NO: 13 - RNA, 21 nt, Artificial Sequence
  Synthetic
ucguacuuaucuuaauccuac

SEQ ID NO: 14 - RNA, 21 nt, Artificial Sequence
  Synthetic
ucguacuuaucuuaauccuac

SEQ ID NO: 15 - RNA, 21 nt, Artificial Sequence
  Synthetic
ucguacuuaucuuaauccuac

SEQ ID NO: 16 - RNA, 21 nt, Artificial Sequence
  Synthetic
gcguaggauuaagauaaguac

SEQ ID NO: 17 - RNA, 21 nt, Artificial Sequence
  Synthetic
ucguacuuaucuuaauccuac

SEQ ID NO: 18 - RNA, 21 nt, Artificial Sequence
  Synthetic
ucguacuuaucuuaauccuac

SEQ ID NO: 19 - RNA, 21 nt, Artificial Sequence
  Synthetic
ucguacuuaucuuaauccuac

SEQ ID NO: 20 - RNA, 21 nt, Artificial Sequence
  Synthetic
ucguacuuaucuuaauccuac

SEQ ID NO: 21 - RNA, 23 nt, Artificial Sequence
  Synthetic
cacaaaaucgguucuacagggua

SEQ ID NO: 22 - DNA, 23 bp, Artificial Sequence
  Synthetic
cacaaaaucggutcuacagggua

SEQ ID NO: 23 - RNA, 13 nt, Artificial Sequence
  Synthetic
cuguggaagucua

SEQ ID NO: 24 - RNA, 13 nt, Artificial Sequence
  Synthetic
cuguggaagucua

SEQ ID NO: 25 - DNA, 20 bp, Artificial Sequence
  Synthetic
agactaggactactactatt

SEQ ID NO: 26 - DNA, 23 bp, Artificial Sequence
  Synthetic
cacaaaaucggutcuacagggua

SEQ ID NO: 27 - DNA, 19 bp, Artificial Sequence
  Synthetic
atagtagtagtcctagtct

SEQ ID NO: 28 - RNA, 23 nt, Artificial Sequence
  Synthetic
cacaaaaucgguucuacagggua

SEQ ID NO: 29 - DNA, 23 bp, Artificial Sequence
  Synthetic
cacaaaaucggutcuacagggua

SEQ ID NO: 30 - RNA, 19 nt, Artificial Sequence
  Synthetic
uucguaguugucuuagucc

SEQ ID NO: 31 - DNA, 19 bp, Artificial Sequence
  Synthetic
atagtagtagtcctagtct